European Patent Application EP 4 678 178 A1, published January 14, 2026. Title: Method for preventing, inhibiting and/or treating cancer metastasis. Applicant: Upadia Holding B.V. The sequence listing filed with the application follows.

SEQUENCE LISTING (12 sequences)

SEQ ID NO: 1 - protein, 8 aa, llama sp
GRTFSTYA

SEQ ID NO: 2 - protein, 8 aa, llama sp
SKGGGITY

SEQ ID NO: 3 - protein, 14 aa, llama sp
DPVSSVAKSPVAYP

SEQ ID NO: 4 - protein, 124 aa, llama sp
EVQLVESGGGLVQAGGSLRLSCAASGRTFSTYAMGWTRQAPGKEREFVAAISKGGGITYYSDSVRGRFTISKENAKNTVYLQMNSLKPEDTAVYYCAADPVSSVAKSPVAYPYWGQGTQVTVSS

SEQ ID NO: 5 - protein, 8 aa, llama sp
GRTFRIND

SEQ ID NO: 6 - protein, 7 aa, llama sp
TSGGNTN

SEQ ID NO: 7 - protein, 14 aa, llama sp
DGLRFDSTRYRPFD

SEQ ID NO: 8 - protein, 123 aa, llama sp
EVQLVESGGGLVQAGGSLRLSCAASGRTFRINDMGWYRQAPGKSRDMVARITSGGNTNYADSVRGRFTISRDNAKNTVYLQMNSLKPEDTAVYYCNADGLRFDSTRYRPFDSWGQGTQVTVSS

SEQ ID NO: 9 - protein, 8 aa, llama sp
GSIRGFVA

SEQ ID NO: 10 - protein, 6 aa, llama sp
TNGGTL

SEQ ID NO: 11 - protein, 9 aa, llama sp
RQIGASGYD

SEQ ID NO: 12 - protein, 117 aa, llama sp
EVQLVESGGGLVQAGGSLRLSCAASGSIRGFVAMAWYRQAPGKQREWVATVTNGGTLYGDSVRGRFTGSRDNAKNTVYLQMNSLKPEDTAVYYCALRQIGASGYDYWGQGTQVTVSS